European Patent Specification EP 3 388 074 B1, published August 23, 2023. Title: Mimotope. Applicant: Affiris AG. The sequence listing filed with the application follows.

SEQUENCE LISTING (57 sequences)

SEQ ID NO: 1 - protein, 8 aa, Artificial
  artificial peptide
DMPVDPDN

SEQ ID NO: 2 - protein, 8 aa, Artificial
  artificial peptide
CDQPVLPD

SEQ ID NO: 3 - protein, 8 aa, Artificial
  artificial peptide
CDMPVLPD

SEQ ID NO: 4 - protein, 8 aa, Artificial
  artificial peptide
CDSPVLPD

SEQ ID NO: 5 - protein, 8 aa, Artificial
  artificial peptide
CDSPVWAE

SEQ ID NO: 6 - protein, 8 aa, Artificial
  artificial peptide
CDTPVLAE

SEQ ID NO: 7 - protein, 9 aa, Artificial
  artificial peptide
CDQPVLPDN

SEQ ID NO: 8 - protein, 9 aa, Artificial
  artificial peptide
CDMPVLPDN

SEQ ID NO: 9 - protein, 9 aa, Artificial
  artificial peptide
CDSPVLPDN

SEQ ID NO: 10 - protein, 9 aa, Artificial
  artificial peptide
CDQPVTAEN

SEQ ID NO: 11 - protein, 9 aa, Artificial
  artificial peptide
CDSPVWAEN

SEQ ID NO: 12 - protein, 9 aa, Artificial
  artificial peptide
CDTPVLAEN

SEQ ID NO: 13 - protein, 9 aa, Artificial
  artificial peptide
CHDRPVTPD

SEQ ID NO: 14 - protein, 8 aa, Artificial
  artificial peptide
CDRPVTPD

SEQ ID NO: 15 - protein, 8 aa, Artificial
  artificial peptide
CDNPVHPE

SEQ ID NO: 16 - protein, 8 aa, Artificial
  artificial peptide
CDVPVLPD

SEQ ID NO: 17 - protein, 8 aa, Artificial
  artificial peptide
CDTPVYPD

SEQ ID NO: 18 - protein, 8 aa, Artificial
  artificial peptide
CDTPVIPD

SEQ ID NO: 19 - protein, 10 aa, Artificial
  artificial peptide
CHDRPVTPDN

SEQ ID NO: 20 - protein, 9 aa, Artificial
  artificial peptide
CDRPVTPDN

SEQ ID NO: 21 - protein, 9 aa, Artificial
  artificial peptide
CDNPVHPEN

SEQ ID NO: 22 - protein, 9 aa, Artificial
  artificial peptide
CDVPVLPDN

SEQ ID NO: 23 - protein, 9 aa, Artificial
  artificial peptide
CDTPVYPDN

SEQ ID NO: 24 - protein, 9 aa, Artificial
  artificial peptide
CDTPVIPDN

SEQ ID NO: 25 - protein, 9 aa, Artificial
  artificial peptide
CDQPVLPDG

SEQ ID NO: 26 - protein, 9 aa, Artificial
  artificial peptide
CDMPVLPDG

SEQ ID NO: 27 - protein, 9 aa, Artificial
  artificial peptide
CDSPVLPDG

SEQ ID NO: 28 - protein, 9 aa, Artificial
  artificial peptide
CDSPVWAEG

SEQ ID NO: 29 - protein, 9 aa, Artificial
  artificial peptide
CDRPVAPEG

SEQ ID NO: 30 - protein, 9 aa, Artificial
  artificial peptide
CDHPVHPDS

SEQ ID NO: 31 - protein, 9 aa, Artificial
  artificial peptide
CDMPVSPDR

SEQ ID NO: 32 - protein, 9 aa, Artificial
  artificial peptide
CDSPVPPDD

SEQ ID NO: 33 - protein, 9 aa, Artificial
  artificial peptide
CDQPVYPDI

SEQ ID NO: 34 - protein, 9 aa, Artificial
  artificial peptide
CDRPVYPDI

SEQ ID NO: 35 - protein, 9 aa, Artificial
  artificial peptide
CDHPVTPDR

SEQ ID NO: 36 - protein, 9 aa, Artificial
  artificial peptide
CEYPVYPES

SEQ ID NO: 37 - protein, 9 aa, Artificial
  artificial peptide
CDTPVLPDS

SEQ ID NO: 38 - protein, 9 aa, Artificial
  artificial peptide
CDMPVTPDT

SEQ ID NO: 39 - protein, 9 aa, Artificial
  artificial peptide
CDAPVTPDT

SEQ ID NO: 40 - protein, 9 aa, Artificial
  artificial peptide
CDSPVVPDN

SEQ ID NO: 41 - protein, 9 aa, Artificial
  artificial peptide
CDLPVTPDR

SEQ ID NO: 42 - protein, 9 aa, Artificial
  artificial peptide
CDSPVHPDT

SEQ ID NO: 43 - protein, 9 aa, Artificial
  artificial peptide
CDAPVRPDS

SEQ ID NO: 44 - protein, 9 aa, Artificial
  artificial peptide
CDMPVWPDG

SEQ ID NO: 45 - protein, 9 aa, Artificial
  artificial peptide
CDAPVYPDG

SEQ ID NO: 46 - protein, 9 aa, Artificial
  artificial peptide
CDRPVQPDR

SEQ ID NO: 47 - protein, 10 aa, Artificial
  artificial peptide
CYDRPVQPDR

SEQ ID NO: 48 - protein, 9 aa, Artificial
  artificial peptide
CDMPVDPEN

SEQ ID NO: 49 - protein, 9 aa, Artificial
  artificial peptide
CDMPVDADN

SEQ ID NO: 50 - protein, 8 aa, Artificial
  artificial peptide
DQPVLPDC

SEQ ID NO: 51 - protein, 8 aa, Artificial
  artificial peptide
DMPVLPDC

SEQ ID NO: 52 - protein, 9 aa, Artificial
  artificial peptide
CEMPVDPDN

SEQ ID NO: 53 - protein, 9 aa, Artificial
  artificial peptide
CDMPVDPDN

SEQ ID NO: 54 - protein, 9 aa, Artificial
  artificial peptide
DMPVDPDNC

SEQ ID NO: 55 - protein, 9 aa, Artificial
  artificial peptide
CDMPVDPGS

SEQ ID NO: 56 - protein, 9 aa, Artificial
  artificial peptide
DMPVDPGSC

SEQ ID NO: 57 - protein, 9 aa, Artificial
  consensus sequence
  MISC_FEATURE (1)..(1): Xaa = (any amino acid residue)n, whereby n = 0 or an integer of more than 0
  MISC_FEATURE (2)..(2): Xaa = an amino acid residue selected from the group consisting of aspartic acid (D) and glutamic acid (E)
  MISC_FEATURE (3)..(3): Xaa = any amino acid residue
  MISC_FEATURE (6)..(6): Xaa = any amino acid residue
  MISC_FEATURE (7)..(7): Xaa = an amino acid residue selected from the group consisting of proline (P) and alanine (A)
  MISC_FEATURE (8)..(8): Xaa = an amino acid residue selected from the group consisting of aspartic acid (D) and glutamic acid (E)
  MISC_FEATURE (9)..(9): Xaa = (any amino acid residue)n, whereby n = 0 or an integer of more than 0
XXXPVXXXX